European Patent Specification EP 3 813 869 B1, published October 18, 2023. Title: METHODS OF INHIBITING CEREBRAL INFLAMMATION. Applicant: UNIVERSITÉ DE GENÈVE; ORION BIOTECHNOLOGY SWITZERLAND SÀRL; HÔPITAUX UNIVERSITAIRES DE GENÈVE. The sequence listing filed with the application follows.

SEQUENCE LISTING (81 sequences)

SEQ ID NO: 1 - protein, 59 aa, Homo sapiens
CCFAYIARPLPRAHIKEYFYTSGKCSNPAVVFVTRKNRQVCANPEKKWVREYINSLEMS

SEQ ID NO: 2 - protein, 10 aa, Artificial Sequence
  synthetic
QGPPLMALQS

SEQ ID NO: 3 - protein, 10 aa, Artificial Sequence
  synthetic
QGPPLMWMQV

SEQ ID NO: 4 - protein, 10 aa, Artificial Sequence
  synthetic
QGPPLMWLQV

SEQ ID NO: 5 - protein, 10 aa, Artificial Sequence
  synthetic
QGPPLMWTQS

SEQ ID NO: 6 - protein, 10 aa, Artificial Sequence
  synthetic
QGPPLMWLQT

SEQ ID NO: 7 - protein, 10 aa, Artificial Sequence
  synthetic
QGPPLMWTQV

SEQ ID NO: 8 - protein, 10 aa, Artificial Sequence
  synthetic
QGPPLMWMQS

SEQ ID NO: 9 - protein, 10 aa, Artificial Sequence
  synthetic
QGPPLMATQS

SEQ ID NO: 10 - protein, 10 aa, Artificial Sequence
  synthetic
QGPPLMWLQS

SEQ ID NO: 11 - protein, 10 aa, Artificial Sequence
  synthetic
QGPPLMALQV

SEQ ID NO: 12 - protein, 10 aa, Artificial Sequence
  synthetic
QGPPLMWLGG

SEQ ID NO: 13 - protein, 10 aa, Artificial Sequence
  synthetic
QGPPLMWRGS

SEQ ID NO: 14 - protein, 10 aa, Artificial Sequence
  synthetic
QGPLLMWLQV

SEQ ID NO: 15 - protein, 10 aa, Artificial Sequence
  synthetic
QGPPLMQTTP

SEQ ID NO: 16 - protein, 10 aa, Artificial Sequence
  synthetic
QGPPGDTVLW

SEQ ID NO: 17 - protein, 10 aa, Artificial Sequence
  synthetic
QGPPGDIVLA

SEQ ID NO: 18 - protein, 10 aa, Artificial Sequence
  synthetic
QGPPGSYDYS

SEQ ID NO: 19 - protein, 10 aa, Artificial Sequence
  synthetic
QGPPGDGGSV

SEQ ID NO: 20 - protein, 10 aa, Artificial Sequence
  synthetic
QGPLSGQSTP

SEQ ID NO: 21 - protein, 10 aa, Artificial Sequence
  synthetic
QGPPGDWLQV

SEQ ID NO: 22 - protein, 10 aa, Artificial Sequence
  synthetic
QGPPLMSFQS

SEQ ID NO: 23 - protein, 10 aa, Artificial Sequence
  synthetic
QGPPLMSTQS

SEQ ID NO: 24 - protein, 10 aa, Artificial Sequence
  synthetic
QGPPLMSLQV

SEQ ID NO: 25 - protein, 10 aa, Artificial Sequence
  synthetic
QGPPLMGLQV

SEQ ID NO: 26 - protein, 10 aa, Artificial Sequence
  synthetic
QGPLSGWLQV

SEQ ID NO: 27 - protein, 10 aa, Artificial Sequence
  synthetic
QGPPLMSVLA

SEQ ID NO: 28 - protein, 10 aa, Artificial Sequence
  synthetic
QGPPGSWSSV

SEQ ID NO: 29 - protein, 10 aa, Artificial Sequence
  synthetic
QGPPLGSMGP

SEQ ID NO: 30 - protein, 10 aa, Artificial Sequence
  synthetic
QGPPLSWLQV

SEQ ID NO: 31 - protein, 10 aa, Artificial Sequence
  synthetic
QGPPLSWLQS

SEQ ID NO: 32 - protein, 10 aa, Artificial Sequence
  synthetic
QGPPGQWSQV

SEQ ID NO: 33 - protein, 10 aa, Artificial Sequence
  synthetic
QGPPMMAGLS

SEQ ID NO: 34 - protein, 10 aa, Artificial Sequence
  synthetic
QGPPLSWQQS

SEQ ID NO: 35 - protein, 10 aa, Artificial Sequence
  synthetic
QGPPGMWSQS

SEQ ID NO: 36 - protein, 10 aa, Artificial Sequence
  synthetic
QGPPLQWRQS

SEQ ID NO: 37 - protein, 10 aa, Artificial Sequence
  synthetic
QGPPLMGTQS

SEQ ID NO: 38 - protein, 10 aa, Artificial Sequence
  synthetic
QGPPLMQLQV

SEQ ID NO: 39 - protein, 10 aa, Artificial Sequence
  synthetic
QGPPLSWSQV

SEQ ID NO: 40 - protein, 10 aa, Artificial Sequence
  synthetic
QGPPMSWSQS

SEQ ID NO: 41 - protein, 10 aa, Artificial Sequence
  synthetic
QGPPLMNLQV

SEQ ID NO: 42 - protein, 10 aa, Artificial Sequence
  synthetic
QGPPMSAYQV

SEQ ID NO: 43 - protein, 10 aa, Artificial Sequence
  synthetic
QGPPMQGGLS

SEQ ID NO: 44 - protein, 10 aa, Artificial Sequence
  synthetic
QGPPLMSLAV

SEQ ID NO: 45 - protein, 10 aa, Artificial Sequence
  synthetic
QGPPLMSLTV

SEQ ID NO: 46 - protein, 10 aa, Artificial Sequence
  synthetic
QGPLSGWAQV

SEQ ID NO: 47 - protein, 10 aa, Artificial Sequence
  synthetic
QGPLSQSSQV

SEQ ID NO: 48 - protein, 10 aa, Artificial Sequence
  synthetic
QGPLSSQSQV

SEQ ID NO: 49 - protein, 10 aa, Artificial Sequence
  synthetic
QGPLGQQGQV

SEQ ID NO: 50 - protein, 10 aa, Artificial Sequence
  synthetic
QGPPLQWFQV

SEQ ID NO: 51 - protein, 10 aa, Artificial Sequence
  synthetic
QGPPLQWTQV

SEQ ID NO: 52 - protein, 10 aa, Artificial Sequence
  synthetic
QGPPLMALSV

SEQ ID NO: 53 - protein, 10 aa, Artificial Sequence
  synthetic
QGPPLMWSQV

SEQ ID NO: 54 - protein, 10 aa, Artificial Sequence
  synthetic
QGPPGQWGQV

SEQ ID NO: 55 - protein, 10 aa, Artificial Sequence
  synthetic
QGPPGSWSQV

SEQ ID NO: 56 - protein, 10 aa, Artificial Sequence
  synthetic
QGPPLMSSQS

SEQ ID NO: 57 - protein, 10 aa, Artificial Sequence
  synthetic
QGPPLMGLSV

SEQ ID NO: 58 - protein, 10 aa, Artificial Sequence
  synthetic
QGPPLMTLQV

SEQ ID NO: 59 - protein, 10 aa, Artificial Sequence
  synthetic
QGPPGQWYQS

SEQ ID NO: 60 - protein, 10 aa, Artificial Sequence
  synthetic
QGPPLQWMQA

SEQ ID NO: 61 - protein, 10 aa, Artificial Sequence
  synthetic
QGPPLQWMQV

SEQ ID NO: 62 - protein, 10 aa, Artificial Sequence
  synthetic
QGPPLMSTQV

SEQ ID NO: 63 - protein, 10 aa, Artificial Sequence
  synthetic
QGPPLMSLSV

SEQ ID NO: 64 - protein, 10 aa, Artificial Sequence
  synthetic
QGPPLMSLQS

SEQ ID NO: 65 - protein, 10 aa, Artificial Sequence
  synthetic
QGPPLMSLQA

SEQ ID NO: 66 - protein, 10 aa, Artificial Sequence
  synthetic
QGPPLMSVQS

SEQ ID NO: 67 - protein, 10 aa, Artificial Sequence
  synthetic
QGPPLMSAQS

SEQ ID NO: 68 - protein, 10 aa, Artificial Sequence
  synthetic
QGPPLMSGQS

SEQ ID NO: 69 - protein, 10 aa, Artificial Sequence
  synthetic
QGPPLMSGQV

SEQ ID NO: 70 - protein, 69 aa, Artificial Sequence
  synthetic
QGPPLMATQSCCFAYIARPLPRAHIKEYFYTSGKCSNPAVVFVTRKNRQVCANPEKKWVREYINSLEMS

SEQ ID NO: 71 - protein, 69 aa, Artificial Sequence [sequence omitted]

SEQ ID NO: 72 - protein, 69 aa, Artificial Sequence
  synthetic
QGPPLMSLQVCCFAYIARPLPRAHIKEYFYTSGKCSNPAVVFVTRKNRQVCANPEKKWVREYINSLEMS

SEQ ID NO: 73 - protein, 69 aa, Artificial Sequence
  Met-RANTES
MSPYSSDTTPCCFAYIARPLPRAHIKEYFYTSGKCSNPAVVFVTRKNRQVCANPEKKWVREYINSLEMS

SEQ ID NO: 74 - protein, 67 aa, Artificial Sequence
  AOP-RANTES
  MISC_FEATURE (1)..(1): N-terminally modified with CH3-(CH2)4-O-N=CH-C(O)-
PYSSDTTPCCFAYIARPLPRAHIKEYFYTSGKCSNPAVVFVTRKNRQVCANPEKKWVREYINSLEMS

SEQ ID NO: 75 - protein, 67 aa, Artificial Sequence; identical to SEQ ID NO: 74
  NNY-RANTES
  MISC_FEATURE (1)..(1): N-terminally modified with CH3-(CH2)7-C(O)-

SEQ ID NO: 76 - protein, 65 aa, Artificial Sequence
  PSC-RANTES
  MISC_FEATURE (1)..(1): N-terminally modified with N(alpha)-(n-nonanoyl)-des-Ser1-[L-thioprolyl2, L-cyclohexylglycyl3]
SSDTTPCCFAYIARPLPRAHIKEYFYTSGKCSNPAVVFVTRKNRQVCANPEKKWVREYINSLEMS

SEQ ID NO: 77 - protein, 68 aa, Artificial Sequence
  pVU5
CPYSSDTTPCCFAYIARPLPRAHIKEYFYTSGKCSNPAVVFVTRKNRQVCANPEKKWVREYINSLEMS

SEQ ID NO: 78 - protein, 68 aa, Artificial Sequence
  pVU14
SPASSDTTPCCFAYIARPLPRAHIKEYFYTSGKCSNPAVVFVTRKNRQVCANPEKKWVREYINSLEMS

SEQ ID NO: 79 - protein, 68 aa, Artificial Sequence
  pVU43
SPYSSDTTPCCFAYIARPLPRAHIKEYFYTSGKCSNPAVVFVTRENRQVCANPEKKWVREYINSLEMS

SEQ ID NO: 80 - protein, 59 aa, Artificial Sequence; identical to SEQ ID NO: 1
  RANTES (9-68)

SEQ ID NO: 81 - protein, 69 aa, Artificial Sequence
  P1
LSPVSSQSSACCFAYIARPLPRAHIKEYFYTSGKCSNPAVVFVTRKNRQVCANPEKKWVREYINSLEMS